European Patent Application EP 4 714 971 A1, published March 25, 2026. Title: ANTIBODY OR ANTIGEN-BINDING FRAGMENT THEREOF, ANTIBODY-DRUG CONJUGATE, AND USE THEREOF. Applicant: SHANGHAI HANSOH BIOMEDICAL CO., LTD. Application IB. The sequence listing filed with the application follows.

SEQUENCE LISTING (72 sequences)

SEQ ID NO: 1 - protein, 994 aa, Homo sapiens
MRPVALLLLPSLLALLAHGLSLEAPTVGKGQAPGIEETDGELTAAPTPEQPERGVHFVTTAPTLKLLNHHPLLEEFLQEGLEKGDEELRPALPFQPDPPAPFTPSPLPRLANQDSRPVFTSPTPAMAAVPTQPQSKEGPWSPESESPMLRITAPLPPGPSMAVPTLGPGEIASTTPPSRAWTPTQEGPGDMGRPWVAEVVSQGAGIGIQGTITSSTASGDDEETTTTTTIITTTITTVQTPGPCSWNFSGPEGSLDSPTDLSSPTDVGLDCFFYISVYPGYGVEIKVQNISLREGETVTVEGLGGPDPLPLANQSFLLRGQVIRSPTHQAALRFQSLPPPAGPGTFHFHYQAYLLSCHFPRRPAYGDVTVTSLHPGGSARFHCATGYQLKGARHLTCLNATQPFWDSKEPVCIAACGGVIRNATTGRIVSPGFPGNYSNNLTCHWLLEAPEGQRLHLHFEKVSLAEDDDRLIIRNGDNVEAPPVYDSYEVEYLPIEGLLSSGKHFFVELSTDSSGAAAGMALRYEAFQQGHCYEPFVKYGNFSSSTPTYPVGTTVEFSCDPGYTLEQGSIIIECVDPHDPQWNETEPACRAVCSGEITDSAGVVLSPNWPEPYGRGQDCIWGVHVEEDKRIMLDIRVLRIGPGDVLTFYDGDDLTARVLGQYSGPRSHFKLFTSMADVTIQFQSDPGTSVLGYQQGFVIHFFEVPRNDTCPELPEIPNGWKSPSQPELVHGTVVTYQCYPGYQVVGSSVLMCQWDLTWSEDLPSCQRVTSCHDPGDVEHSRRLISSPKFPVGATVQYICDQGFVLMGSSILTCHDRQAGSPKWSDRAPKCLLEQLKPCHGLSAPENGARSPEKQLHPAGATIHFSCAPGYVLKGQASIKCVPGHPSHWSDPPPICRAASLDGFYNSRSLDVAKAPAASSTLDAAHIAAAIFLPLVAMVLLVGGVYFYFSRLQGKSSLQLPRPRPRPYNRITIESAFDNPTYETGSLSFAGDERI

SEQ ID NO: 2 - protein, 996 aa, Macaca fascicularis
MRPAALLLLPSLLALLAHGLSSEAPTMGKGQAPGIEETDGELTAAPTPEQPERGVHFVTTAPTLKLLNHHPLLEEFLQEGLEKGDEELRPALPFQPDPPTPFTPSPLPRLANQDSRPVFTSPTPATAAVPTQPQSKEGPWSLESEPPVLRITAPLPPGPSMAVPTLRPGERPSTTPPSRAWTPTQEGPGDMGRPWVPEVVSQGAGIGIQGTIASSTASGDDEETTTTTTTTIITTTITTVQTPGPCSWNFSGPEGSLDSPTDLSSPPDVGLDCFFYISVYPGYGVEIKVQNISLREGETVTVEGLGGPDPLPLANQSFLLRGQVIRSPTHQAALRFQSLPPPAGPGTFHFHYQAYLLSCHFPHRPAYGDVTVTSLHPGGSARFHCATGYQLKGARHLTCLNATQPFWDSKEPVCIAACGGVIRNATTGRIVSPGFPGNYSNNLTCHWLLEAPEGQRLHLHFEKVSLAEDDDRLIIRNGDNVEAPPVYDSYEVEYLPIEGLLSSGKHFFVELSTDSSGAAAGMALRYEAFQQGHCYEPFVKYGNFSSSAPTYPVGTTVEFSCDPGYTLEQGSIIIECVDPHDPQWNETEPACRAVCSGEITDSAGVVLSPNWPEPYGRGQDCIWGVHVEEDKRIMLDVRVLRIGPGDVLTFYDGDDLTARVLGQYSGPHSHFKLFTSMADVTIQFQSDPGTSVLGYQQGFVIHFFEVPRNDTCPELPEIPNGWKSPSQPDLVHGTVVTYQCYPGYQVVGSSVLMCQWDLTWSEDLPSCQRVTSCHDPGDVEHSRRLISSPKFPVGATVQYICDQGFVLTGTSILTCHDRQAGSPKWSDRAPKCLLEQLKPCHGLSAPENGARSPEKRLHPAGATIHFSCAPGYVLKGQASIKCVPGHPSHWSDPPPICKAASLDGFYNSRSLDVAKAPAASSTLDAAHIAAAIFLPLVAMVLLVGGVYFYFSRLQGKSSLQLPRTRPRPYNRITVESAFDNPTYETGSLSFAGDERI

SEQ ID NO: 3 - protein, 991 aa, Mus musculus
MRPAALLLLPSLLALLAHGLSSEAPITGEGHATGIRETDGELTAAPTPEQSDRGVHFVTTAPTLKLLNHHPLLEEFLQEGLEREEAPQPALPFQPDSPTHFTPSPLPRLTNQDNRPVFTSPTPAVAAAPTQPHSREKPWNLESKPPELSITSSLPPGPSMAVPTLLPEDRPSTTPPSQAWTPTQEGPGDMDRPWVPEVMSKTTGLGVEGTIATSTASGDDEETTTTIITTTVTTVQPPGPCSWNFSGPEGSLDSPTAPSSPSDVGLDCFYYISVYPGYGVEIKVENISLQEGETITVEGLGGPDPLPLANQSFLLRGQVIRSPTHQAALRFQSLPLPAGPGTFHFRYQAYLLSCHFPRRPAYGDVTVTSLHPGGSAHFHCATGYQLKGARFLTCLNATQPFWDSQEPVCIAACGGVIRNATTGRIVSPGFPGNYSNNLTCHWLLEAPESQRLHLHFEKVSLAEDDDRLIIRNGNNVEAPPVYDSYEVEYLPIEGLLSSGRHFFVEFSTDSSGAAAGMALRYEAFQQGHCYEPFVKYGNFSSSAPSYPVGTTVEFSCDPGYTLEQGSIIIECVDLHDPQWNETEPACRAVCSGEITDSAGVVLSPNWPEPYGRGQDCIWGVHVEEDKRIMLDIRVLRIGSGDVLTFYDGDDLTARVLGQYSGPRGHFKLFTSMADVTIQFQSDPGTSALGYQQGFVIHFFEVPRNDTCPELPEIPNGWKNPSQPELVHGTVVTYQCYPGYQVVGSSILMCQWDLSWSEDLPSCQRVTSCHDPGDVEHSRRLISSPKFPVGATVQYVCDQGFVLTGSAILTCHDRQAGSPKWSDRAPKCLLEQFKPCHGLSAPENGARSPEKRLHPAGATIHFSCAPGYVLKGQASIKCVPGHPSHWSDPPPICRAASLDGFYNGRSLDVAKAPAASSALDAAHLAAAIFLPLVAMVLLVGGVYLYFSRFQGKSPLQLPRTHPRPYNRITVESAFDNPTYETGSLSFAGDERI

SEQ ID NO: 4 - protein, 1024 aa, Homo sapiens
MPAARPPAAGLRGISLFLALLLGSPAAALERDALPEGDASPLGPYLLPSGAPERGSPGKEHPEERVVTAPPSSSQSAEVLGELVLDGTAPSAHHDIPALSPLLPEEARPKHALPPKKKLPSLKQVNSARKQLRPKATSAATVQRAGSQPASQGLDLLSSSTEKPGPPGDPDPIVASEEASEVPLWLDRKESAVPTTPAPLQISPFTSQPYVAHTLPQRPEPGEPGPDMAQEAPQEDTSPMALMDKGENELTGSASEESQETTTSTIITTTVITTEQAPALCSVSFSNPEGYIDSSDYPLLPLNNFLECTYNVTVYTGYGVELQVKSVNLSDGELLSIRGVDGPTLTVLANQTLLVEGQVIRSPTNTISVYFRTFQDDGLGTFQLHYQAFMLSCNFPRRPDSGDVTVMDLHSGGVAHFHCHLGYELQGAKMLTCINASKPHWSSQEPICSAPCGGAVHNATIGRVLSPSYPENTNGSQFCIWTIEAPEGQKLHLHFERLLLHDKDRMTVHSGQTNKSALLYDSLQTESVPFEGLLSEGNTIRIEFTSDQARAASTFNIRFEAFEKGHCYEPYIQNGNFTTSDPTYNIGTIVEFTCDPGHSLEQGPAIIECINVRDPYWNDTEPLCRAMCGGELSAVAGVVLSPNWPEPYVEGEDCIWKIHVGEEKRIFLDIQFLNLSNSDILTIYDGDEVMPHILGQYLGNSGPQKLYSSTPDLTIQFHSDPAGLIFGKGQGFIMNYIEVSRNDSCSDLPEIQNGWKTTSHTELVRGARITYQCDPGYDIVGSDTLTCQWDLSWSSDPPFCEKIMYCTDPGEVDHSTRLISDPVLLVGTTIQYTCNPGFVLEGSSLLTCYSRETGTPIWTSRLPHCVSEESLACDNPGLPENGYQILYKRLYLPGESLTFMCYEGFELMGEVTIRCILGQPSHWNGPLPVCKVNQDSFEHALEVAEAAAETSLEGGNMALAIFIPVLIISLLLGGAYIYITRCRYYSNLRLPLMYSHPYSQITVETEFDNPIYETGETREYEVSI

SEQ ID NO: 5 - protein, 910 aa, Homo sapiens
MGTPRAQHPPPPQLLFLILLSCPWIQGLPLKEEEILPEPGSETPTVASEALAELLHGALLRRGPEMGYLPGSDRDPTLATPPAGQTLAVPSLPRATEPGTGPLTTAVTPNGVRGAGPTAPELLTPPPGTTAPPPPSPASPGPPLGPEGGEEETTTTIITTTTVTTTVTSPVLCNNNISEGEGYVESPDLGSPVSRTLGLLDCTYSIHVYPGYGIEIQVQTLNLSQEEELLVLAGGGSPGLAPRLLANSSMLGEGQVLRSPTNRLLLHFQSPRVPRGGGFRIHYQAYLLSCGFPPRPAHGDVSVTDLHPGGTATFHCDSGYQLQGEETLICLNGTRPSWNGETPSCMASCGGTIHNATLGRIVSPEPGGAVGPNLTCRWVIEAAEGRRLHLHFERVSLDEDNDRLMVRSGGSPLSPVIYDSDMDDVPERGLISDAQSLYVELLSETPANPLLLSLRFEAFEEDRCFAPFLAHGNVTTTDPEYRPGALATFSCLPGYALEPPGPPNAIECVDPTEPHWNDTEPACKAMCGGELSEPAGVVLSPDWPQSYSPGQDCVWGVHVQEEKRILLQVEILNVREGDMLTLFDGDGPSARVLAQLRGPQPRRRLLSSGPDLTLQFQAPPGPPNPGLGQGFVLHFKEVPRNDTCPELPPPEWGWRTASHGDLIRGTVLTYQCEPGYELLGSDILTCQWDLSWSAAPPACQKIMTCADPGEIANGHRTASDAGFPVGSHVQYRCLPGYSLEGAAMLTCYSRDTGTPKWSDRVPKCALKYEPCLNPGVPENGYQTLYKHHYQAGESLRFFCYEGFELIGEVTITCVPGHPSQWTSQPPLCKVTQTTDPSRQLEGGNLALAILLPLGLVIVLGSGVYIYYTKLQGKSLFGFSGSHSYSPITVESDFSNPLYEAGDTREYEVSI

SEQ ID NO: 6 - protein, 445 aa, synthetic construct
EVQLVQSGAEVKKPGESLKISCKGSGYSFTSSWINWVRQMPGKGLEWMGRIYPGEGDTNYNGNFEGQVTISADKSISTAYLQWSSLKASDTAMYYCTRGLVMDYWGQGTLVTVSSASTKGPSVFPLAPSSKSTSGGTAALGCLVKDYFPEPVTVSWNSGALTSGVHTFPAVLQSSGLYSLSSVVTVPSSSLGTQTYICNVNHKPSNTKVDKKVEPKSCDKTHTCPPCPAPELLGGPSVFLFPPKPKDTLMISRTPEVTCVVVDVSHEDPEVKFNWYVDGVEVHNAKTKPREEQYNSTYRVVSVLTVLHQDWLNGKEYKCKVSNKALPAPIEKTISKAKGQPREPQVYTLPPSREEMTKNQVSLTCLVKGFYPSDIAVEWESNGQPENNYKTTPPVLDSDGSFFLYSKLTVDKSRWQQGNVFSCSVMHEALHNHYTQKSLSLSPGK

SEQ ID NO: 7 - protein, 218 aa, synthetic construct
EIVLTQSPATLSLSPGERATLSCRASQSVDYNGISYMHWYQQKPGQAPRLLIYAASNVQSGIPARFSGSGSGTDFTLTISSLEPEDFAVYYCQQSIEDPPTFGGGTKVEIKRTVAAPSVFIFPPSDEQLKSGTASVVCLLNNFYPREAKVQWKVDNALQSGNSQESVTEQDSKDSTYSLSSTLTLSKADYEKHKVYACEVTHQGLSSPVTKSFNRGEC

SEQ ID NO: 8 - protein, 116 aa, Mus musculus
QVQLQQSGAELVRPGASVTLSCKASGYTFTGYEMHWVKQTPVHGLEWIGGIDPETDNTVYNQKFKGKAILTEDKSSSTAYMELRRLTSEDSAVYYCTRGDWYFDIWGTGTTVTVSS

SEQ ID NO: 9 - protein, 112 aa, Mus musculus
DIVLSQSPSSQAVSVGEKVTMSCKSSQSLLNSRTRENYLAWYQQKPGQSPKLLIYWASTRESGVPDRFTGSGSGTDFTLTISSVQAEDLAVYYCQQSYNLFTFGSGTILEIK

SEQ ID NO: 10 - protein, 116 aa, Mus musculus
QVQLQQSGAELARPGASVTLSCKASGYKFTDYEMHWVKETPVNGLEWIGGIDPETENTVYNQKFKVKAILTEDKSSRTAYMELRSLTSEDSAVYYCTRGDWYFDVWGTGTTVTVSS

SEQ ID NO: 11 - protein, 112 aa, Mus musculus
DIVMSQSPSSQAVSVGEKVTMSCKSSQSLLNSRTRENYLAWYQQKAGQSPKLLIYWASTRDSGVPDRFTGSGSGTAFTLTINSVQAEDLAVYYCKQSYNLFTFGSGTKLEIK

SEQ ID NO: 12 - protein, 116 aa, Mus musculus
QVQLQQSGAELARPGASVTLSCKASGYTFTDYEMHWVKETPVDGLEWIGGIDPETDNTVYNQKFKVKAILTEDKSSRIAYMELRSLTSEDSAVYYCTRGDWYFDVWGTGTTVTVSS

SEQ ID NO: 13 - protein, 112 aa, Mus musculus
DIVMSQSPSSQAVSVGEKVTMSCKSSQSLLNSRTRENYLAWYQQKAGQSPKLLIYWASTRDSGVPDRFTGSGSGTDFTLTINSVQAEDLAVYYCKQSYNLFTFGSGTKLEIK

SEQ ID NO: 14 - protein, 116 aa, Mus musculus
QVQLQQSGAELVRPGASVTLSCKASGYTFTDYEMHWVRQTPVHGLEWIGGIDPESDNTVYNQKFKGKVTLTEDKSSSTAYMEFRSLTSEDSAVYYCTRGDWYFDVWGTGTTVTVSS

SEQ ID NO: 15 - protein, 112 aa, Mus musculus
DIVMSQSPSSQAVSVGEKVTMTCKSSQSLLNSRTRENYLAWYQQKPGQSPKLLIYWASTRESGVPDRFTGSGSGADFTLTISSVQAEDLAVYYCGQSYNLFTFGSGTKLEIK

SEQ ID NO: 16 - protein, 118 aa, Mus musculus
QVQLQQPGAELVKPGASVKLSCKASGYTFSIYWMHWVKQRPGQGLEWIGMIHPNSGSTNYNEKFKSKATLTVDKSSSTAYMQLSSLTSEDSAVYYCARGGNYVAMDYWGQGTSVTVSS

SEQ ID NO: 17 - protein, 107 aa, Mus musculus
QIVLTQSPAIMSASLGERVTMTCTASSSVSSSYLHWYQQKPGSSPKLWIYSTSNLASGVPARFSGSGSGTSYSLTISSMEAEDAATYYCHQYHRSLTFGSGTKLEIK

SEQ ID NO: 18 - protein, 119 aa, Mus musculus
DVQLQESGPGLVKPSQSLSLTCSVTGQSITSGYFWNWIRQLPGNKLEWMGHIRYDGNNNYNPSLKNRVSITRDTSKNQFFLKLNSVTTEDTATYYCARWLLRYYAMDSWGQGTSVTVSS

SEQ ID NO: 19 - protein, 112 aa, Mus musculus
DVVMTQTPLTLSVIIGQPASISCKSSQSLLDSDGKTYLNWLLQRPGHSPKRLIYLVSKLDSGVPDRFTGSGSGTDFTLKISRVEAEDLGVYYCWQGTHFPWTFGGGTKLEIK

SEQ ID NO: 20 - protein, 116 aa, Mus musculus
QVQLQQSGAELARPGASVKMSCKASGYTFTSYTMHWVKQRPGQGLEWIGYINPRSDYTKYNQKVKDKATLTADKSSSTAYMQLSSLTSEDSAVYYCARGGLGLDYWGQGTTLTVSS

SEQ ID NO: 21 - protein, 107 aa, Mus musculus
DIQMTQSPSSLSASLGERVSLTCRASQEISGYLSWLQQTPDGTIKRLIYAASTLHSGVPKRFSGSRSGSDYSLTISSLESEDFAGYYCLQYASYPYTFGGGTKLEIK

SEQ ID NO: 22 - protein, 116 aa, Mus musculus
QVQLQQSGAELARPGASVKMSCKASGYTFTSYTMHWVKQRPGQGLEWIGYINPSSDYTKYNQKFKGKATMTADKSSSTAYMQLSSLTSEDSAVYYCGRGLVPFAYWGQGTLVTVSA

SEQ ID NO: 23 - protein, 107 aa, Mus musculus
DIQMTQSPSSLSASLGERVSLTCRASQEISGYLIWLQQKPDGTIKRLIYAASTLDSGVPKRVSGSRSGSDYSLTISSLESEDFADYYCLQYASYPLTFGGGTKLELK

SEQ ID NO: 24 - protein, 120 aa, Mus musculus
QVQLQQSGPELMKPGASVKISCKASGYTFTDYYINWMKQRPGQGLEWIGWIFPGSDNPYYNEMFKDKATVSVDKSSSAVFMLLTSLTSEDSAVYFCARGRYYGLYTMDYWGQGTSVTVSS

SEQ ID NO: 25 - protein, 107 aa, Mus musculus
DIQMTQTTSSLSASLGDRVTISCRASQDIRNYLNWYQQKADGTVKFLIYYTSRLHSGVPSRFSGSGSGTDFSLTISNLEQEDVATYFCQQGNTLPWTFGGGTKVEIK

SEQ ID NO: 26 - protein, 125 aa, Lama glama
EVQLVESGGGSVQPGGSLRLSCEASGLTYNKDCMAWFRQAPGKEREGVAIINGVGRTRYADSVKGRFTISKDNAKNTLYLQMNNLKPEDTAMYYCAAQRASSSCGSLSRAWYDYWGRGTQVTVSS

SEQ ID NO: 27 - protein, 124 aa, Lama glama
HVQLVESGGGSVQAGGSLRLSCAVSGFTSSRGWMAWFRQAPGKEREGVAVIGRRSGDIYYADSLKGRFTISHDSTENTLYLQMNNLKPEDTATYYCAVGDQAGHVLTSSPYRYWGQGTQVTVSS

SEQ ID NO: 28 - protein, 124 aa, Lama glama
DVQLVESGGGSVQAGGSLRVSCAVSGYTKSSGWMGWFRQAPGKEREGVAAIGRRSGDRYYVDSVKGRFTISLDSTKNTLYLQMNDLKPEDTGTYYCAAGGRAGNVLTSQPYRYWGQGTQVTVSS

SEQ ID NO: 29 - protein, 116 aa, synthetic construct
QVQLVQSGAEVKKPGASVKVSCKASGYTFTDYEMHWVRQAPGQGLEWMGGIDPESDNTVYNQKFKGRVTLTEDTSTSTAYMELRSLRSEDTAVYYCTRGDWYFDVWGQGTTVTVSS

SEQ ID NO: 30 - protein, 112 aa, synthetic construct
DIVMTQSPDSLAVSLGERATINCKSSQSLLNSRTRENYLAWYQQKPGQPPKLLIYWASTRESGVPDRFSGSGSGTDFTLTISSLQAEDVAVYYCGQSYNLFTFGQGTKLEIK

SEQ ID NO: 31 - protein, 118 aa, synthetic construct
EVQLVQSGAEVKKPGSSVKVSCKASGYTFSIYWMHWVRQAPGQGLEWIGMIHPNSGSTNYNEKFKSRATLTVDKSTSTAYMELSSLRSEDTAVYYCARGGNYVAMDYWGQGTLVTVSS

SEQ ID NO: 32 - protein, 107 aa, synthetic construct
DIQMTQSPSSLSASVGDRVTITCTASSSVSSSYLHWYQQKPGKAPKLLIYSTSNLASGVPSRFSGSGSGTDFTLTISSLQPEDFATYYCHQYHRSLTFGGGTKVEIK

SEQ ID NO: 33 - protein, 330 aa, Homo sapiens
ASTKGPSVFPLAPSSKSTSGGTAALGCLVKDYFPEPVTVSWNSGALTSGVHTFPAVLQSSGLYSLSSVVTVPSSSLGTQTYICNVNHKPSNTKVDKKVEPKSCDKTHTCPPCPAPELLGGPSVFLFPPKPKDTLMISRTPEVTCVVVDVSHEDPEVKFNWYVDGVEVHNAKTKPREEQYNSTYRVVSVLTVLHQDWLNGKEYKCKVSNKALPAPIEKTISKAKGQPREPQVYTLPPSREEMTKNQVSLTCLVKGFYPSDIAVEWESNGQPENNYKTTPPVLDSDGSFFLYSKLTVDKSRWQQGNVFSCSVMHEALHNHYTQKSLSLSPGK

SEQ ID NO: 34 - protein, 107 aa, synthetic construct
DIQLTQSPSSLSASVGDRVTMTCTASSSVSSSYLHWYQQKPGKSPKLWIYSTSNLASGVPSRFSGSGSGTDYTLTISSLQPEDFATYYCHQYHRSLTFGGGTKVEIK

SEQ ID NO: 35 - protein, 120 aa, synthetic construct
EVQLVQSGAEVKKPGASVKISCKASGYTFTDYYINWMRQAPGQGLEWIGWIFPGSDNPYYNEMFKDRVTVTVDKSTSTVYMELSSLRSEDTAVYFCARGRYYGLYTMDYWGQGTLVTVSS

SEQ ID NO: 36 - protein, 107 aa, synthetic construct
DIQMTQSPSSLSASVGDRVTITCRASQDIRNYLNWYQQKPGKAPKFLIYYTSRLHSGVPSRFSGSGSGTDFTLTISSLQPEDFATYYCQQGNTLPWTFGGGTKVEIK

SEQ ID NO: 37 - protein, 5 aa, Mus musculus
DYEMH

SEQ ID NO: 38 - protein, 17 aa, Mus musculus
GIDPESDNTVYNQKFKG

SEQ ID NO: 39 - protein, 7 aa, Mus musculus
GDWYFDV

SEQ ID NO: 40 - protein, 17 aa, Mus musculus
KSSQSLLNSRTRENYLA

SEQ ID NO: 41 - protein, 7 aa, Mus musculus
WASTRES

SEQ ID NO: 42 - protein, 8 aa, Mus musculus
GQSYNLFT

SEQ ID NO: 43 - protein, 5 aa, Mus musculus
IYWMH

SEQ ID NO: 44 - protein, 17 aa, Mus musculus
MIHPNSGSTNYNEKFKS

SEQ ID NO: 45 - protein, 9 aa, Mus musculus
GGNYVAMDY

SEQ ID NO: 46 - protein, 12 aa, Mus musculus
TASSSVSSSYLH

SEQ ID NO: 47 - protein, 7 aa, Mus musculus
STSNLAS

SEQ ID NO: 48 - protein, 8 aa, Mus musculus
HQYHRSLT

SEQ ID NO: 49 - protein, 5 aa, Mus musculus
DYYIN

SEQ ID NO: 50 - protein, 17 aa, Mus musculus
WIFPGSDNPYYNEMFKD

SEQ ID NO: 51 - protein, 11 aa, Mus musculus
GRYYGLYTMDY

SEQ ID NO: 52 - protein, 11 aa, Mus musculus
RASQDIRNYLN

SEQ ID NO: 53 - protein, 7 aa, Mus musculus
YTSRLHS

SEQ ID NO: 54 - protein, 9 aa, Mus musculus
QQGNTLPWT

SEQ ID NO: 55 - protein, 446 aa, synthetic construct
QVQLVQSGAEVKKPGASVKVSCKASGYTFTDYEMHWVRQAPGQGLEWMGGIDPESDNTVYNQKFKGRVTLTEDTSTSTAYMELRSLRSEDTAVYYCTRGDWYFDVWGQGTTVTVSSASTKGPSVFPLAPSSKSTSGGTAALGCLVKDYFPEPVTVSWNSGALTSGVHTFPAVLQSSGLYSLSSVVTVPSSSLGTQTYICNVNHKPSNTKVDKKVEPKSCDKTHTCPPCPAPELLGGPSVFLFPPKPKDTLMISRTPEVTCVVVDVSHEDPEVKFNWYVDGVEVHNAKTKPREEQYNSTYRVVSVLTVLHQDWLNGKEYKCKVSNKALPAPIEKTISKAKGQPREPQVYTLPPSREEMTKNQVSLTCLVKGFYPSDIAVEWESNGQPENNYKTTPPVLDSDGSFFLYSKLTVDKSRWQQGNVFSCSVMHEALHNHYTQKSLSLSPGK

SEQ ID NO: 56 - protein, 219 aa, synthetic construct
DIVMTQSPDSLAVSLGERATINCKSSQSLLNSRTRENYLAWYQQKPGQPPKLLIYWASTRESGVPDRFSGSGSGTDFTLTISSLQAEDVAVYYCGQSYNLFTFGQGTKLEIKRTVAAPSVFIFPPSDEQLKSGTASVVCLLNNFYPREAKVQWKVDNALQSGNSQESVTEQDSKDSTYSLSSTLTLSKADYEKHKVYACEVTHQGLSSPVTKSFNRGEC

SEQ ID NO: 57 - protein, 448 aa, synthetic construct
EVQLVQSGAEVKKPGSSVKVSCKASGYTFSIYWMHWVRQAPGQGLEWIGMIHPNSGSTNYNEKFKSRATLTVDKSTSTAYMELSSLRSEDTAVYYCARGGNYVAMDYWGQGTLVTVSSASTKGPSVFPLAPSSKSTSGGTAALGCLVKDYFPEPVTVSWNSGALTSGVHTFPAVLQSSGLYSLSSVVTVPSSSLGTQTYICNVNHKPSNTKVDKKVEPKSCDKTHTCPPCPAPELLGGPSVFLFPPKPKDTLMISRTPEVTCVVVDVSHEDPEVKFNWYVDGVEVHNAKTKPREEQYNSTYRVVSVLTVLHQDWLNGKEYKCKVSNKALPAPIEKTISKAKGQPREPQVYTLPPSREEMTKNQVSLTCLVKGFYPSDIAVEWESNGQPENNYKTTPPVLDSDGSFFLYSKLTVDKSRWQQGNVFSCSVMHEALHNHYTQKSLSLSPGK

SEQ ID NO: 58 - protein, 214 aa, synthetic construct
DIQMTQSPSSLSASVGDRVTITCTASSSVSSSYLHWYQQKPGKAPKLLIYSTSNLASGVPSRFSGSGSGTDFTLTISSLQPEDFATYYCHQYHRSLTFGGGTKVEIKRTVAAPSVFIFPPSDEQLKSGTASVVCLLNNFYPREAKVQWKVDNALQSGNSQESVTEQDSKDSTYSLSSTLTLSKADYEKHKVYACEVTHQGLSSPVTKSFNRGEC

SEQ ID NO: 59 - protein, 107 aa, Homo sapiens [sequence omitted]

SEQ ID NO: 60 - protein, 214 aa, synthetic construct
DIQLTQSPSSLSASVGDRVTMTCTASSSVSSSYLHWYQQKPGKSPKLWIYSTSNLASGVPSRFSGSGSGTDYTLTISSLQPEDFATYYCHQYHRSLTFGGGTKVEIKRTVAAPSVFIFPPSDEQLKSGTASVVCLLNNFYPREAKVQWKVDNALQSGNSQESVTEQDSKDSTYSLSSTLTLSKADYEKHKVYACEVTHQGLSSPVTKSFNRGEC

SEQ ID NO: 61 - protein, 450 aa, synthetic construct
EVQLVQSGAEVKKPGASVKISCKASGYTFTDYYINWMRQAPGQGLEWIGWIFPGSDNPYYNEMFKDRVTVTVDKSTSTVYMELSSLRSEDTAVYFCARGRYYGLYTMDYWGQGTLVTVSSASTKGPSVFPLAPSSKSTSGGTAALGCLVKDYFPEPVTVSWNSGALTSGVHTFPAVLQSSGLYSLSSVVTVPSSSLGTQTYICNVNHKPSNTKVDKKVEPKSCDKTHTCPPCPAPELLGGPSVFLFPPKPKDTLMISRTPEVTCVVVDVSHEDPEVKFNWYVDGVEVHNAKTKPREEQYNSTYRVVSVLTVLHQDWLNGKEYKCKVSNKALPAPIEKTISKAKGQPREPQVYTLPPSREEMTKNQVSLTCLVKGFYPSDIAVEWESNGQPENNYKTTPPVLDSDGSFFLYSKLTVDKSRWQQGNVFSCSVMHEALHNHYTQKSLSLSPGK

SEQ ID NO: 62 - protein, 214 aa, synthetic construct
DIQMTQSPSSLSASVGDRVTITCRASQDIRNYLNWYQQKPGKAPKFLIYYTSRLHSGVPSRFSGSGSGTDFTLTISSLQPEDFATYYCQQGNTLPWTFGGGTKVEIKRTVAAPSVFIFPPSDEQLKSGTASVVCLLNNFYPREAKVQWKVDNALQSGNSQESVTEQDSKDSTYSLSSTLTLSKADYEKHKVYACEVTHQGLSSPVTKSFNRGEC

SEQ ID NO: 63 - protein, 125 aa, synthetic construct
EVQLVESGGGLVQPGGSLRLSCAASGFTFSKDCMAWFRQAPGKGREGVAIISGVGRTRYADSVKGRFTISRDNAKNSLYLQMNSLRAEDTAVYYCAAQRASSSCGSLSRAWYDYWGRGTLVTVSS

SEQ ID NO: 64 - protein, 124 aa, synthetic construct
HVQLVESGGGLVQPGGSLRLSCAVSGFTSSRGWMAWFRQAPGKEREGVAVIGRRSGDIYYADSLKGRFTISHDNAKNSLYLQMNSLRAEDTATYYCAVGDQAGHVLTSSPYRYWGQGTMVTVSS

SEQ ID NO: 65 - protein, 5 aa, Lama glama
KDCMA

SEQ ID NO: 66 - protein, 16 aa, Lama glama
IISGVGRTRYADSVKG

SEQ ID NO: 67 - protein, 17 aa, Lama glama
QRASSSCGSLSRAWYDY

SEQ ID NO: 68 - protein, 5 aa, Lama glama
RGWMA

SEQ ID NO: 69 - protein, 17 aa, Lama glama
VIGRRSGDIYYADSLKG

SEQ ID NO: 70 - protein, 15 aa, Lama glama
GDQAGHVLTSSPYRY

SEQ ID NO: 71 - protein, 357 aa, synthetic construct
EVQLVESGGGLVQPGGSLRLSCAASGFTFSKDCMAWFRQAPGKGREGVAIISGVGRTRYADSVKGRFTISRDNAKNSLYLQMNSLRAEDTAVYYCAAQRASSSCGSLSRAWYDYWGRGTLVTVSSEPKSSDKTHTCPPCPAPELLGGPSVFLFPPKPKDTLMISRTPEVTCVVVDVSHEDPEVKFNWYVDGVEVHNAKTKPREEQYNSTYRVVSVLTVLHQDWLNGKEYKCKVSNKALPAPIEKTISKAKGQPREPQVYTLPPSREEMTKNQVSLTCLVKGFYPSDIAVEWESNGQPENNYKTTPPVLDSDGSFFLYSKLTVDKSRWQQGNVFSCSVMHEALHNHYTQKSLSLSPGK

SEQ ID NO: 72 - protein, 356 aa, synthetic construct
HVQLVESGGGLVQPGGSLRLSCAVSGFTSSRGWMAWFRQAPGKEREGVAVIGRRSGDIYYADSLKGRFTISHDNAKNSLYLQMNSLRAEDTATYYCAVGDQAGHVLTSSPYRYWGQGTMVTVSSEPKSSDKTHTCPPCPAPELLGGPSVFLFPPKPKDTLMISRTPEVTCVVVDVSHEDPEVKFNWYVDGVEVHNAKTKPREEQYNSTYRVVSVLTVLHQDWLNGKEYKCKVSNKALPAPIEKTISKAKGQPREPQVYTLPPSREEMTKNQVSLTCLVKGFYPSDIAVEWESNGQPENNYKTTPPVLDSDGSFFLYSKLTVDKSRWQQGNVFSCSVMHEALHNHYTQKSLSLSPGK